European Patent Application EP 4 219 550 A1, published August 2, 2023. Title: MONOCLONAL ANTIBODIES TO ELTD1 AND USES THEREOF. Applicant: OKLAHOMA MEDICAL RESEARCH FOUNDATION. Application EP. The sequence listing filed with the application follows.

SEQUENCE LISTING (123 sequences)

SEQ ID NO: 1 - DNA, 756 bp, synthetic construct
  misc_feature 1..756: note = Synthetic primer
  source 1..756: mol_type = other DNA
gccctgactcagccgtcctcggtgtcagcaaacccgggagaaaccgtcaagatcacctgctccgggagtagtggcagctactatggctggcaccagcagaagtctcctggcagtgcccctgtcactctgatctatgacaacaccaacagaccctcggacatcccttcacgattcttcggttccaaatccggttccacagccacattaaccatcactggggtccaagccgacgacgaggctgtctattactgtgggagctgggacagcagcagtggtgctggtatatttggggccgggacaaccctgaccgtcctaggtcagtcctctagatcttccagcggtggtggcagctccggtggtggcggttccgccgtgacgttggacgagtccgggggcggcctccagacgcccggaggagcgctcagcctcgtctgcaaggcctccgggttcaccttcagcagttacgccatgaactgggtgcgacaggcgcccggcaaggggctggagtgggtcgcagctattagcagtgatggtagtagcacaggatatgggccggcggtggagggccgtgccaccatctcgagggacaacgggcagagcacagtgaggctgcagctgaacaacctcagggctgaggacaccggcacctactactgcgccaaaaatgcttgtacttacggtagtggttattgtggttggagtggtgctggtggtatcgacgcatggggccacgggaccgaagtcatcgtctcctcc

SEQ ID NO: 2 - protein, 105 aa, synthetic construct
  REGION 1..105: note = Synthetic peptide
ALTQPSSVSANPGETVKITCSGSSGSYYGWHQQKSPGSAPVTLIYDNTNRPSDIPSRFFGSKSGSTATLTITGVQADDEAVYYCGSWDSSSGAGIFGAGTTLTVL

SEQ ID NO: 3 - protein, 18 aa, synthetic construct
  REGION 1..18: note = Synthetic peptide
GQSSRSSSGGGSSGGGGS

SEQ ID NO: 4 - protein, 129 aa, synthetic construct
  REGION 1..129: note = Synthetic peptide
AVTLDESGGGLQTPGGALSLVCKASGFTFSSYAMNWVRQAPGKGLEWVAAISSDGSSTGYGPAVEGRATISRDNGQSTVRLQLNNLRAEDTGTYYCAKNACTYGSGYCGWSGAGGIDAWGHGTEVIVSS

SEQ ID NO: 5 - DNA, 741 bp, synthetic construct
  misc_feature 1..741: note = Synthetic primer
  source 1..741: mol_type = other DNA
gccctgactcagccgtcctcggcgtcagcaaacccgggagaaaccgtcgagatcacctgctccgggggttacagcggctatggctggttccagcagaagtctcctggcagtgcccctgtcactctgatctatgaaaacgacaagagaccctcggacatcccttcacgattctccggttccaaatccggctccacgggcacattaaccatcactggggtccaagccgacgacgaggctgtctatttctgtgggagtgcagacaggagtaataatgtgggtatatttggggccgggacaaccctgaccgtcctaggtcagtcctctagatcttccggcggtggtggcagctccggtggtggcggttccgccgtgacgttggacgagtccgggggcggcctccagacgcccggaggagcgctcagcctcgtctgcaaggcctccgggttcgacttcagcagttacgccatgaactgggtgcgacaggcgcccggcaaggggctggagtgggtcgctgctattagtgacactggtagtggcacaggatacggggcggcggtgaagggccgtgccaccatctcgagggacaacgggcagagcacagtgaggctgcagctgaacaacctcagggcagaggacaccggcatctacttctgcgccaaagatgctggttatgctgctggttggggtgctgctgggagcatcgacgcatggggccacgggaccgaagtcatcgtctcctcc

SEQ ID NO: 6 - protein, 109 aa, synthetic construct
  REGION 1..109: note = Synthetic peptide
DVAQAALTQPSSASANPGETVEITCSGGYSGYGWFQQKSPGSAPVTLIYENDKRPSDIPSRFSGSKSGSTGTLTITGVQADDEAVYFCGSADRSNNVGIFGAGTTLTVL

SEQ ID NO: 7 - protein, 18 aa, synthetic construct
  REGION 1..18: note = Synthetic peptide
GQSSRSSGGGGSSGGGGS

SEQ ID NO: 8 - protein, 125 aa, synthetic construct
  REGION 1..125: note = Synthetic peptide
AVTLDESGGGLQTPGGALSLVCKASGFDFSSYAMNWVRQAPGKGLEWVAAISDTGSGTGYGAAVKGRATISRDNGQSTVRLQLNNLRAEDTGIYFCAKDAGYAAGWGAAGSIDAWGHGTEVIVSS

SEQ ID NO: 9 - DNA, 738 bp, synthetic construct
  misc_feature 1..738: note = Synthetic primer
  source 1..738: mol_type = other DNA
gccctgactcagccgtcctcggtgtcagcaaacctgggaggaaccgtcaagatcacctgctccgggggtagtggcagctacggctggttccagcagaaggcacctggcagtgcccctgtcactctgatctatgacaacaccaacagaccctcgaacatcccttcacgattctccggttccacatctggctccacaagcacattagccatcactggggtccaagccgacgacgaggctgtctattactgtgggagtgaagacatcagctatatcggtatatttggggccgggacaaccctgaccgtcctaggtcagtcctctagatcttccggcggtggtggcagctccggtggtggcggttccgccgtgacgttggacgagtccgggggcggcctccagacgcccggaggagggctcagcctcgtctgcaaggcctccggcttcaccttcagcagtttctacatgttctgggtgcgccaggcgcccggcaaggggctggaatacgtcgcagctattagcaacactggtagtggcacagactacggggcggcggtgcagggccgtgccaccatctcgagggacaacgggcagagcacagtgaggctgcagctgaacaacctcagggctgaggacaccgccacctactactgcgccaaagctgctgctggttgtactggttgtggtggtgctggtagtatcgacgcatggggccacgggaccgaagtcatcgtctcctcc

SEQ ID NO: 10 - protein, 103 aa, synthetic construct
  REGION 1..103: note = Synthetic peptide
ALTQPSSVSANLGGTVKITCSGGSGSYGWFQQKAPGSAPVTLIYDNTNRPSNIPSRFSGSTSGSTSTLAITGVQADDEAVYYCGSEDISYIGIFGAGTTLTVL

SEQ ID NO: 11 - protein, 18 aa, synthetic construct
  REGION 1..18: note = Synthetic peptide
GQSSRSSGGGGSSGGGGS

SEQ ID NO: 12 - protein, 125 aa, synthetic construct
  REGION 1..125: note = Synthetic peptide
AVTLDESGGGLQTPGGGLSLVCKASGFTFSSFYMFWVRQAPGKGLEYVAAISNTGSGTDYGAAVQGRATISRDNGQSTVRLQLNNLRAEDTATYYCAKAAAGCTGCGGAGSIDAWGHGTEVIVSS

SEQ ID NO: 13 - DNA, 741 bp, synthetic construct
  misc_feature 1..741: note = Synthetic primer
  source 1..741: mol_type = other DNA
gccctgactcagccgtcctcggtgtcagcaaacccaggagaaaccgtcaagatcacctgctctgggggcagctatagctatggctggtaccagcagaaggcacctggcagtgcccctgtcactgtgatctatgacaacaccaacagaccctcgaacatcccttcacgattctccggttccacatccggctccacagccacattaaccatcactggggtccgagccgaggacgaggctgtctattactgtgggagtgcagacagcagttacattggtatatttggggccgggacaaccctgaccgtcctaggtcagtcctctagatcttccggcggtggtggcagctccggtggtggcggttccgccgtgacgttggacgagtccgggggcggcctccagacgcccggaggaacgctcagcctcgtctgcaaggcctccgggttcaccttcagcagcgtcaacatgttctggatgcgacaggctccaggcaaggggctggagttcgttgctgctattggcaatgatgctggtggcacagactacggggcggcggtggatggccgtgccaccatctcgagggacaacgggcagagcacagtgaggctgcagctgaacaacctcagggctgaggacaccgccacctactactgcgccaaagcttctgcttgtagtacttctggttgtggtggtgctggtagcatcgacgcatggggccacgggaccgaagtcatcgtctcctcc

SEQ ID NO: 14 - protein, 103 aa, synthetic construct
  REGION 1..103: note = Synthetic peptide
ALTQPSSVSANPGETVKITCSGGSYSYGWYQQKAPGSAPVTVIYDNTNRPSNIPSRFSGSTSGSTATLTITGVRAEDEAVYYCGSADSSYIGIFGAGTTLTVL

SEQ ID NO: 15 - protein, 18 aa, synthetic construct
  REGION 1..18: note = Synthetic peptide
GQSSRSSGGGGSSGGGGS

SEQ ID NO: 16 - protein, 126 aa, synthetic construct
  REGION 1..126: note = Synthetic peptide
AVTLDESGGGLQTPGGTLSLVCKASGFTFSSVNMFWMRQAPGKGLEFVAAIGNDAGGTDYGAAVDGRATISRDNGQSTVRLQLNNLRAEDTATYYCAKASACSTSGCGGAGSIDAWGHGTEVIVSS

SEQ ID NO: 17 - DNA, 741 bp, synthetic construct
  misc_feature 1..741: note = Synthetic primer
  source 1..741: mol_type = other DNA
gccctgactcagccgtcctcggtgtcagcaaacctgggaggaaccgtcaagatcatctgctccgggggtggtggcagctatggctggttccagcagaaggcacctggcagtgcccctgtcactgtgatctatgacaacaacaagagaccctcggacatcccttcacgattctccggttccaaatccggctccacggccacattaaccatcactggggtccgagccgaggacgaggctgtctattactgtgggagtgcagacaacacctatgttggtatatttggggccgggacaaccctgaccgtcctaggtcagtcctctagatcttccagcggtggtggcagctccggtggtggcggttccgccgtgacgttggacgagtccgggggcggcctccagacgcccggaggaacgctcagcctcgtctgcaaggcctccgggttcaccttcagcagcgtcaacatgttctggatgcgacaggctccaggcaaggggctggggttcgttgctgctattggcaatgatgctggtggcacagactacggggcggcggtggatggccgtgccaccatctcgagggacaacgggcagagcacagtgaggctgcagctgaacaacctcagggctgaggacaccgccacctactactgcgccaaagcttctgcttgtagtacctctggttgtggtggtgctggtagcatcgacgcatggggccacgggaccgaagtcatcgtctcctcc

SEQ ID NO: 18 - protein, 103 aa, synthetic construct
  REGION 1..103: note = Synthetic peptide
ALTQPSSVSANLGGTVKIICSGGGGSYGWFQQKAPGSAPVTVIYDNNKRPSDIPSRFSGSKSGSTATLTITGVRAEDEAVYYCGSADNTYVGIFGAGTTLTVL

SEQ ID NO: 19 - protein, 18 aa, synthetic construct
  REGION 1..18: note = Synthetic peptide
GQSSRSSSGGGSSGGGGS

SEQ ID NO: 20 - protein, 126 aa, synthetic construct
  REGION 1..126: note = Synthetic peptide
AVTLDESGGGLQTPGGTLSLVCKASGFTFSSVNMFWMRQAPGKGLGFVAAIGNDAGGTDYGAAVDGRATISRDNGQSTVRLQLNNLRAEDTATYYCAKASACSTSGCGGAGSIDAWGHGTEVIVSS

SEQ ID NO: 21 - DNA, 744 bp, synthetic construct
  misc_feature 1..744: note = Synthetic primer
  source 1..744: mol_type = other DNA
gccctgactcagccgtcctcggtgtcagcaaacccaggagaaaccgtcaagatcacctgctccgggggtggcagctatggttatggctggtaccagcagaaggcacctagcagtgcccctgtcactgtgatttgctgggataacaagagaccctcgaacatcccttcacgattctccggttccacatctggctccacagccacattaaccatcactggggtccaagccgaggacgaggctgtctatttctgtgggagtgcagacagcagcggtactgctgctatatttggggccgggacaaacctgaccgtcctaggtcagtcctctagatcttccagcggtggtggcagctccggtggtggcggttccgccgtgacgttggacgagtccgggggcggcctccagacgcccggaggagcgctcagcctcatctgcaaggcctccgggttcgacttcagcagttacgccatgaactgggtgcgacaggcgcccggcaaggggctggagtgggtcgcaagtattgatgatggtggtagtgacacaacctacggggcggcggtgaagggccgcgccaccgtctcgagggacaacgggcagagcacagtgaggctgcagttgaacaacctcagggctgaggacaccggcacctactactgcgccaaagatgctagtagtggtggtgtttggagtgctgctgctggcatcgacgcatggggccacgggaccgaagtcatcgtctcctcc

SEQ ID NO: 22 - protein, 105 aa, synthetic construct
  REGION 1..105: note = Synthetic peptide
ALTQPSSVSANPGETVKITCSGGGSYGYGWYQQKAPSSAPVTVICWDNKRPSNIPSRFSGSTSGSTATLTITGVQAEDEAVYFCGSADSSGTAAIFGAGTNLTVL

SEQ ID NO: 23 - protein, 18 aa, synthetic construct
  REGION 1..18: note = Synthetic peptide
GQSSRSSSGGGSSGGGGS

SEQ ID NO: 24 - protein, 125 aa, synthetic construct
  REGION 1..125: note = Synthetic peptide
AVTLDESGGGLQTPGGALSLICKASGFDFSSYAMNWVRQAPGKGLEWVASIDDGGSDTTYGAAVKGRATVSRDNGQSTVRLQLNNLRAEDTGTYYCAKDASSGGVWSAAAGIDAWGHGTEVIVSS

SEQ ID NO: 25 - protein, 9 aa, synthetic construct
  REGION 1..9: note = Synthetic peptide
SGSSGSYYG

SEQ ID NO: 26 - protein, 7 aa, synthetic construct
  REGION 1..7: note = Synthetic peptide
DNTNRPS

SEQ ID NO: 27 - protein, 11 aa, synthetic construct
  REGION 1..11: note = Synthetic peptide
GSWDSSSGAGI

SEQ ID NO: 28 - protein, 5 aa, synthetic construct
  REGION 1..5: note = Synthetic peptide
SYAMN

SEQ ID NO: 29 - protein, 18 aa, synthetic construct
  REGION 1..18: note = Synthetic peptide
AAISSDGSSTGYGPAVEG

SEQ ID NO: 30 - protein, 20 aa, synthetic construct
  REGION 1..20: note = Synthetic peptide
NACTYGSGYCGWSGAGGIDA

SEQ ID NO: 31 - protein, 8 aa, synthetic construct
  REGION 1..8: note = Synthetic peptide
SGGYSGYG

SEQ ID NO: 32 - protein, 7 aa, synthetic construct
  REGION 1..7: note = Synthetic peptide
ENDKRPS

SEQ ID NO: 33 - protein, 11 aa, synthetic construct
  REGION 1..11: note = Synthetic peptide
GSADRSNNVGI

SEQ ID NO: 34 - protein, 5 aa, synthetic construct
  REGION 1..5: note = Synthetic peptide
SYAMN

SEQ ID NO: 35 - protein, 17 aa, synthetic construct
  REGION 1..17: note = Synthetic peptide
AISDTGSGTGYGAAVKG

SEQ ID NO: 36 - protein, 16 aa, synthetic construct
  REGION 1..16: note = Synthetic peptide
DAGYAAGWGAAGSIDA

SEQ ID NO: 37 - protein, 8 aa, synthetic construct
  REGION 1..8: note = Synthetic peptide
SGGSGSYG

SEQ ID NO: 38 - protein, 7 aa, synthetic construct
  REGION 1..7: note = Synthetic peptide
DNTNRPS

SEQ ID NO: 39 - protein, 10 aa, synthetic construct
  REGION 1..10: note = Synthetic peptide
GSEDISYIGI

SEQ ID NO: 40 - protein, 5 aa, synthetic construct
  REGION 1..5: note = Synthetic peptide
SFYMF

SEQ ID NO: 41 - protein, 17 aa, synthetic construct
  REGION 1..17: note = Synthetic peptide
AISNTGSGTDYGAAVQG

SEQ ID NO: 42 - protein, 16 aa, synthetic construct
  REGION 1..16: note = Synthetic peptide
AAAGCTGCGGAGSIDA

SEQ ID NO: 43 - protein, 8 aa, synthetic construct
  REGION 1..8: note = Synthetic peptide
SGGSYSYG

SEQ ID NO: 44 - protein, 7 aa, synthetic construct
  REGION 1..7: note = Synthetic peptide
DNTNRPS

SEQ ID NO: 45 - protein, 10 aa, synthetic construct
  REGION 1..10: note = Synthetic peptide
GSADSSYIGI

SEQ ID NO: 46 - protein, 5 aa, synthetic construct
  REGION 1..5: note = Synthetic peptide
SVNMF

SEQ ID NO: 47 - protein, 17 aa, synthetic construct
  REGION 1..17: note = Synthetic peptide
AIGNDAGGTDYGAAVDG

SEQ ID NO: 48 - protein, 17 aa, synthetic construct
  REGION 1..17: note = Synthetic peptide
ASACSTSGCGGAGSIDA

SEQ ID NO: 49 - protein, 8 aa, synthetic construct
  REGION 1..8: note = Synthetic peptide
SGGGGSYG

SEQ ID NO: 50 - protein, 7 aa, synthetic construct
  REGION 1..7: note = Synthetic peptide
DNNKRPS

SEQ ID NO: 51 - protein, 10 aa, synthetic construct
  REGION 1..10: note = Synthetic peptide
GSADNTYVGI

SEQ ID NO: 52 - protein, 5 aa, synthetic construct
  REGION 1..5: note = Synthetic peptide
SVNMF

SEQ ID NO: 53 - protein, 17 aa, synthetic construct
  REGION 1..17: note = Synthetic peptide
AIGNDAGGTDYGAAVDG

SEQ ID NO: 54 - protein, 17 aa, synthetic construct
  REGION 1..17: note = Synthetic peptide
ASACSTSGCGGAGSIDA

SEQ ID NO: 55 - protein, 9 aa, synthetic construct
  REGION 1..9: note = Synthetic peptide
SGGGSYGYG

SEQ ID NO: 56 - protein, 7 aa, synthetic construct
  REGION 1..7: note = Synthetic peptide
WDNKRPS

SEQ ID NO: 57 - protein, 11 aa, synthetic construct
  REGION 1..11: note = Synthetic peptide
GSADSSGTAAI

SEQ ID NO: 58 - protein, 5 aa, synthetic construct
  REGION 1..5: note = Synthetic peptide
SYAMN

SEQ ID NO: 59 - protein, 17 aa, synthetic construct
  REGION 1..17: note = Synthetic peptide
SIDDGGSDTTYGAAVKG

SEQ ID NO: 60 - protein, 16 aa, synthetic construct
  REGION 1..16: note = Synthetic peptide
DASSGGVWSAAAGIDA

SEQ ID NO: 61 - protein, 4 aa, synthetic construct
  REGION 1..4: note = Synthetic peptide
GSYG

SEQ ID NO: 62 - protein, 3 aa, synthetic construct
  REGION 1..3: note = Synthetic peptide
WDN

SEQ ID NO: 63 - protein, 11 aa, synthetic construct
  REGION 1..11: note = Synthetic peptide
GSADSSGTAAI

SEQ ID NO: 64 - protein, 8 aa, synthetic construct
  REGION 1..8: note = Synthetic peptide
GFDFSSYA

SEQ ID NO: 65 - protein, 8 aa, synthetic construct
  REGION 1..8: note = Synthetic peptide
IDDGGSDT

SEQ ID NO: 66 - protein, 18 aa, synthetic construct
  REGION 1..18: note = Synthetic peptide
AKDASSGGVWSAAAGIDA

SEQ ID NO: 67 - protein, 9 aa, synthetic construct
  REGION 1..9: note = Synthetic peptide
SGGGSYGYG

SEQ ID NO: 68 - protein, 7 aa, synthetic construct
  REGION 1..7: note = Synthetic peptide
WDNKRPS

SEQ ID NO: 69 - protein, 11 aa, synthetic construct
  REGION 1..11: note = Synthetic peptide
GSADSSGTAAI

SEQ ID NO: 70 - protein, 7 aa, synthetic construct
  REGION 1..7: note = Synthetic peptide
GFDFSSY

SEQ ID NO: 71 - protein, 6 aa, synthetic construct
  REGION 1..6: note = Synthetic peptide
DDGGSD

SEQ ID NO: 72 - protein, 16 aa, synthetic construct
  REGION 1..16: note = Synthetic peptide
DASSGGVWSAAAGIDA

SEQ ID NO: 73 - protein, 4 aa, synthetic construct
  REGION 1..4: note = Synthetic peptide
SGSY

SEQ ID NO: 74 - protein, 3 aa, synthetic construct
  REGION 1..3: note = Synthetic peptide
DNT

SEQ ID NO: 75 - protein, 13 aa, synthetic construct
  REGION 1..13: note = Synthetic peptide
GSWDSSSGAGIFG

SEQ ID NO: 76 - protein, 8 aa, synthetic construct
  REGION 1..8: note = Synthetic peptide
GFTFSSYA

SEQ ID NO: 77 - protein, 8 aa, synthetic construct
  REGION 1..8: note = Synthetic peptide
ISSDGSST

SEQ ID NO: 78 - protein, 22 aa, synthetic construct
  REGION 1..22: note = Synthetic peptide
AKNACTYGSGYCGWSGAGGIDA

SEQ ID NO: 79 - protein, 9 aa, synthetic construct
  REGION 1..9: note = Synthetic peptide
SGSSGSYYG

SEQ ID NO: 80 - protein, 7 aa, synthetic construct
  REGION 1..7: note = Synthetic peptide
DNTNRPS

SEQ ID NO: 81 - protein, 11 aa, synthetic construct
  REGION 1..11: note = Synthetic peptide
GSWDSSSGAGI

SEQ ID NO: 82 - protein, 7 aa, synthetic construct
  REGION 1..7: note = Synthetic peptide
GFTFSSY

SEQ ID NO: 83 - protein, 6 aa, synthetic construct
  REGION 1..6: note = Synthetic peptide
SSDGSS

SEQ ID NO: 84 - protein, 20 aa, synthetic construct
  REGION 1..20: note = Synthetic peptide
NACTYGSGYCGWSGAGGIDA

SEQ ID NO: 85 - protein, 3 aa, synthetic construct
  REGION 1..3: note = Synthetic peptide
YSG

SEQ ID NO: 86 - protein, 3 aa, synthetic construct
  REGION 1..3: note = Synthetic peptide
END

SEQ ID NO: 87 - protein, 13 aa, synthetic construct
  REGION 1..13: note = Synthetic peptide
GSADRSNNVGIFG

SEQ ID NO: 88 - protein, 10 aa, synthetic construct
  REGION 1..10: note = Synthetic peptide
GFDFSSYAMN

SEQ ID NO: 89 - protein, 9 aa, synthetic construct
  REGION 1..9: note = Synthetic peptide
AISDTGSGT

SEQ ID NO: 90 - protein, 18 aa, synthetic construct
  REGION 1..18: note = Synthetic peptide
AKDAGYAAGWGAAGSIDA

SEQ ID NO: 91 - protein, 8 aa, synthetic construct
  REGION 1..8: note = Synthetic peptide
GFTFSSFY

SEQ ID NO: 92 - protein, 8 aa, synthetic construct
  REGION 1..8: note = Synthetic peptide
ISNTGSGT

SEQ ID NO: 93 - protein, 18 aa, synthetic construct
  REGION 1..18: note = Synthetic peptide
AKAAAGCTGCGGAGSIDA

SEQ ID NO: 94 - protein, 8 aa, synthetic construct
  REGION 1..8: note = Synthetic peptide
SGGSGSYG

SEQ ID NO: 95 - protein, 7 aa, synthetic construct
  REGION 1..7: note = Synthetic peptide
DNTNRPS

SEQ ID NO: 96 - protein, 7 aa, synthetic construct
  REGION 1..7: note = Synthetic peptide
DNTNRPS

SEQ ID NO: 97 - protein, 7 aa, synthetic construct
  REGION 1..7: note = Synthetic peptide
GFTFSSF

SEQ ID NO: 98 - protein, 6 aa, synthetic construct
  REGION 1..6: note = Synthetic peptide
SNTGSG

SEQ ID NO: 99 - protein, 16 aa, synthetic construct
  REGION 1..16: note = Synthetic peptide
AAAGCTGCGGAGSIDA

SEQ ID NO: 100 - protein, 3 aa, synthetic construct
  REGION 1..3: note = Synthetic peptide
SYS

SEQ ID NO: 101 - protein, 3 aa, synthetic construct
  REGION 1..3: note = Synthetic peptide
DNT

SEQ ID NO: 102 - protein, 10 aa, synthetic construct
  REGION 1..10: note = Synthetic peptide
GSADSSYIGI

SEQ ID NO: 103 - protein, 8 aa, synthetic construct
  REGION 1..8: note = Synthetic peptide
GFTFSSVN

SEQ ID NO: 104 - protein, 8 aa, synthetic construct
  REGION 1..8: note = Synthetic peptide
IGNDAGGT

SEQ ID NO: 105 - protein, 19 aa, synthetic construct
  REGION 1..19: note = Synthetic peptide
AKASACSTSGCGGAGSIDA

SEQ ID NO: 106 - protein, 8 aa, synthetic construct
  REGION 1..8: note = Synthetic peptide
SGGSYSYG

SEQ ID NO: 107 - protein, 7 aa, synthetic construct
  REGION 1..7: note = Synthetic peptide
DNTNRPS

SEQ ID NO: 108 - protein, 10 aa, synthetic construct
  REGION 1..10: note = Synthetic peptide
GSADSSYIGI

SEQ ID NO: 109 - protein, 7 aa, synthetic construct
  REGION 1..7: note = Synthetic peptide
GFTFSSV

SEQ ID NO: 110 - protein, 6 aa, synthetic construct
  REGION 1..6: note = Synthetic peptide
GNDAGG

SEQ ID NO: 111 - protein, 17 aa, synthetic construct
  REGION 1..17: note = Synthetic peptide
ASACSTSGCGGAGSIDA

SEQ ID NO: 112 - protein, 3 aa, synthetic construct
  REGION 1..3: note = Synthetic peptide
GGS

SEQ ID NO: 113 - protein, 3 aa, synthetic construct
  REGION 1..3: note = Synthetic peptide
DNN

SEQ ID NO: 114 - protein, 10 aa, synthetic construct
  REGION 1..10: note = Synthetic peptide
GSADNTYVGI

SEQ ID NO: 115 - protein, 8 aa, synthetic construct
  REGION 1..8: note = Synthetic peptide
GFTFSSVN

SEQ ID NO: 116 - protein, 8 aa, synthetic construct
  REGION 1..8: note = Synthetic peptide
IGNDAGGT

SEQ ID NO: 117 - protein, 19 aa, synthetic construct
  REGION 1..19: note = Synthetic peptide
AKASACSTSGCGGAGSIDA

SEQ ID NO: 118 - protein, 8 aa, synthetic construct
  REGION 1..8: note = Synthetic peptide
SGGGGSYG

SEQ ID NO: 119 - protein, 7 aa, synthetic construct
  REGION 1..7: note = Synthetic peptide
DNNKRPS

SEQ ID NO: 120 - protein, 10 aa, synthetic construct
  REGION 1..10: note = Synthetic peptide
GSADNTYVGI

SEQ ID NO: 121 - protein, 7 aa, synthetic construct
  REGION 1..7: note = Synthetic peptide
GFTFSSV

SEQ ID NO: 122 - protein, 6 aa, synthetic construct
  REGION 1..6: note = Synthetic peptide
GNDAGG

SEQ ID NO: 123 - protein, 17 aa, synthetic construct
  REGION 1..17: note = Synthetic peptide
ASACSTSGCGGAGSIDA